European Patent Specification EP 3 849 608 B1, published August 30, 2023. Title: NOVEL LILRB4 ANTIBODIES AND USES THEREOF. Applicant: THE BOARD OF REGENTS OF THE UNIVERSITY OF TEXAS IMMUNE-ONC THERAPEUTICS, INC. The sequence listing filed with the application follows.

SEQUENCE LISTING (238 sequences)

SEQ ID NO: 1 - protein, 123 aa, Artificial sequence
  Synthetic amino acid
EQSLEESGGLEESGGRLVTPGTPLTLTCTASGFTINSAHMSWVRQAPGKGLEWIGFSTTGGPSYYANWAKGRFTISRTSTTVDLEITSPTIEDTATYFCARDGPGNNIDMDLWGQGTLVTITS

SEQ ID NO: 2 - protein, 8 aa, Artificial sequence
  Synthetic amino acid
GFTINSAH

SEQ ID NO: 3 - protein, 7 aa, Artificial sequence
  Synthetic amino acid
STTGGPS

SEQ ID NO: 4 - protein, 13 aa, Artificial sequence
  Synthetic amino acid
ARDGPGNNIDMDL

SEQ ID NO: 5 - protein, 110 aa, Artificial sequence
  Synthetic amino acid
ELDLTQTPASVSEPVGGTVTIKCQASQNRGGSIAWYQQKPGQPPKLLIYSASTLASGVPSRFSGSGYGTEFTLTISGVQCADAGTYYCQSTIYSISDIGAFGGGTEVVVK

SEQ ID NO: 6 - protein, 6 aa, Artificial sequence
  Synthetic amino acid
QNRGGS

SEQ ID NO: 7 - protein, 12 aa, Artificial sequence
  Synthetic amino acid
QSTIYSISDIGA

SEQ ID NO: 8 - protein, 115 aa, Artificial sequence
  Synthetic amino acid
QSVEESGGRLVTPGTPLTLTCTVSGIDLTNYAINWVRQAPGEGLEYIGTITGSSNTFYASWAKGRFTISKTSTTVDLKITSPTTEDTGTYFCASNPDSHNANGVWGQGTLVTVSS

SEQ ID NO: 9 - protein, 8 aa, Artificial sequence
  Synthetic amino acid
GIDLTNYA

SEQ ID NO: 10 - protein, 7 aa, Artificial sequence
  Synthetic amino acid
ITGSSNT

SEQ ID NO: 11 - protein, 12 aa, Artificial sequence
  Synthetic amino acid
ASNPDSHNANGV

SEQ ID NO: 12 - protein, 112 aa, Artificial sequence
  Synthetic amino acid
ELVMTQTPASVSEPVEGTVTIKCQASQSVYDNNLAWYQQKPGQPPKLLIYSASTLASGVPSRFSGSGYGTEFTLTISGVECADAATYYCQSYGITNKNNYNSFGGGTEVVVK

SEQ ID NO: 13 - protein, 7 aa, Artificial sequence
  Synthetic amino acid
QSVYDNN

SEQ ID NO: 14 - protein, 13 aa, Artificial sequence
  Synthetic amino acid
QSYGITNKNNYNS

SEQ ID NO: 15 - protein, 121 aa, Artificial sequence
  Synthetic amino acid
EQSVEESGGDLVKPGASLTLTCAASGFSFSSTYCMCWVRQAPGKGLEWIACIHGVSTNNRWYASWPKGRFTISKTSSTTVTLQMTSLTAADTATYFCARSDTDYEWGLSLWGPGTLVTISS

SEQ ID NO: 16 - protein, 9 aa, Artificial sequence
  Synthetic amino acid
GFSFSSTYC

SEQ ID NO: 17 - protein, 9 aa, Artificial sequence
  Synthetic amino acid
IHGVSTNNR

SEQ ID NO: 18 - protein, 13 aa, Artificial sequence
  Synthetic amino acid
ARSDTDYEWGLSL

SEQ ID NO: 19 - protein, 108 aa, Artificial sequence
  Synthetic amino acid
ELDLTQTPASVSEPVGGTVTIKCQASESIGSRLAWYQQKPGQRPKLLIYKASTLASGVPSRFSGSGSGTEFTLTVSDLECADVAAYYCQCAGQSSTWAFGGGTEVEIK

SEQ ID NO: 20 - protein, 6 aa, Artificial sequence
  Synthetic amino acid
ESIGSR

SEQ ID NO: 21 - protein, 10 aa, Artificial sequence
  Synthetic amino acid
QCAGQSSTWA

SEQ ID NO: 22 - protein, 121 aa, Artificial sequence; identical to SEQ ID NO: 15
  Synthetic amino acid

SEQ ID NO: 23 - protein, 9 aa, Artificial sequence
  Synthetic amino acid
GFSFSSTYC

SEQ ID NO: 24 - protein, 9 aa, Artificial sequence
  Synthetic amino acid
IHGVSTNNR

SEQ ID NO: 25 - protein, 13 aa, Artificial sequence
  Synthetic amino acid
ARSDTDYEWGLSL

SEQ ID NO: 26 - protein, 108 aa, Artificial sequence
  Synthetic amino acid
ELVMTQTPASVEAVVGGTVTIKCQASESIGSRLAWYQQKPGQRPKLLIYKASTLASGVPSRFSGSGSGTEFTLTVSDLECADVAAYYCQCAGQSSTWAFGGGTEVVVK

SEQ ID NO: 27 - protein, 6 aa, Artificial sequence
  Synthetic amino acid
ESIGSR

SEQ ID NO: 28 - protein, 10 aa, Artificial sequence
  Synthetic amino acid
QCAGQSSTWA

SEQ ID NO: 29 - protein, 120 aa, Artificial sequence
  Synthetic amino acid
QSVKESGGRLVTPGTPLTLTCTVSGFSLSNNGMSWVRQAPGKGLEWIGIIYVGSGTTDYATWAKGRFTISRTSTTVDLKMTSLTTEDTATYLCARGFGVGDWQEWFFDLWGPGTLVTISS

SEQ ID NO: 30 - protein, 8 aa, Artificial sequence
  Synthetic amino acid
GFSLSNNG

SEQ ID NO: 31 - protein, 8 aa, Artificial sequence
  Synthetic amino acid
IYVGSGTT

SEQ ID NO: 32 - protein, 16 aa, Artificial sequence
  Synthetic amino acid
ARGFGVGDWQEWFFDL

SEQ ID NO: 33 - protein, 108 aa, Artificial sequence
  Synthetic amino acid
ELVMTQTPASVSEPVGGTVTIKCQASESISNYLSWYQQKPGQPPKLLIYKASTLASGVSSRFKGSGSGTEFTLTISDLECADAATYYCQAYWGTSTMAFGGGTEVEIN

SEQ ID NO: 34 - protein, 6 aa, Artificial sequence
  Synthetic amino acid
ESISNY

SEQ ID NO: 35 - protein, 10 aa, Artificial sequence
  Synthetic amino acid
QAYWGTSTMA

SEQ ID NO: 36 - protein, 120 aa, Artificial sequence
  Synthetic amino acid
QSLEESGGRLVTPGTPLTLTCTVSGFSLSNNGMSWVRQAPGKGLEWIGIIYVGSGTTDYASWPKGRFTISRTSTTVDLKMTSLTTEDTATYLCARGFGVGDWQEWFFDLWGPGTLVTVSS

SEQ ID NO: 37 - protein, 8 aa, Artificial sequence
  Synthetic amino acid
GFSLSNNG

SEQ ID NO: 38 - protein, 8 aa, Artificial sequence
  Synthetic amino acid
IYVGSGTT

SEQ ID NO: 39 - protein, 16 aa, Artificial sequence
  Synthetic amino acid
ARGFGVGDWQEWFFDL

SEQ ID NO: 40 - protein, 108 aa, Artificial sequence; identical to SEQ ID NO: 33
  Synthetic amino acid

SEQ ID NO: 41 - protein, 6 aa, Artificial sequence
  Synthetic amino acid
ESISNY

SEQ ID NO: 42 - protein, 10 aa, Artificial sequence
  Synthetic amino acid
QAYWGTSTMA

SEQ ID NO: 43 - protein, 114 aa, Artificial sequence
  Synthetic amino acid
SSVEESGGRLVTPGTPLTLTCTVSGFSLSSYAMAWVRQAPGKGLEWIGIIGTGTTTYYATWVNGRFTISKTSTTVDLKMTSLTTEDTATYFCVRNDVYWAFNLWGQGTLVTVSS

SEQ ID NO: 44 - protein, 8 aa, Artificial sequence
  Synthetic amino acid
GFSLSSYA

SEQ ID NO: 45 - protein, 7 aa, Artificial sequence
  Synthetic amino acid
IGTGTTT

SEQ ID NO: 46 - protein, 11 aa, Artificial sequence
  Synthetic amino acid
VRNDVYWAFNL

SEQ ID NO: 47 - protein, 112 aa, Artificial sequence
  Synthetic amino acid
ELVMTQTPAPVSAAVGGTVTINCQASQSVVNNNALSWYQQKPGQPPKLLIYKASTLASGVPSRFKGSGSGAQFTLTISGVQCDDAATYYCQGGYYIGISDYPFGGGTEVVVK

SEQ ID NO: 48 - protein, 8 aa, Artificial sequence
  Synthetic amino acid
QSVVNNNA

SEQ ID NO: 49 - protein, 12 aa, Artificial sequence
  Synthetic amino acid
QGGYYIGISDYP

SEQ ID NO: 50 - protein, 114 aa, Artificial sequence; identical to SEQ ID NO: 43
  Synthetic amino acid

SEQ ID NO: 51 - protein, 8 aa, Artificial sequence
  Synthetic amino acid
GFSLSSYA

SEQ ID NO: 52 - protein, 7 aa, Artificial sequence
  Synthetic amino acid
IGTGTTT

SEQ ID NO: 53 - protein, 11 aa, Artificial sequence
  Synthetic amino acid
VRNDVYWAFNL

SEQ ID NO: 54 - protein, 112 aa, Artificial sequence
  Synthetic amino acid
ELDLTQTPSSVSAAVGGTVSISCQSSQSVVNNNALSWYQQKPGQPPKLLIYKASTLASGVPSRFKGSGSGAQFTLTISGVQCDDAATYYCQGGYYIGISDYPFGGGTEVEIK

SEQ ID NO: 55 - protein, 8 aa, Artificial sequence
  Synthetic amino acid
QSVVNNNA

SEQ ID NO: 56 - protein, 12 aa, Artificial sequence
  Synthetic amino acid
QGGYYIGISDYP

SEQ ID NO: 57 - protein, 115 aa, Artificial sequence
  Synthetic amino acid
EQSVEESGGGLVTPGGTLTLTCTASGFSISTYAMIWVRQAPGEGLEYIGCIGTGGSAFYAIWAKGRFTISRTSTTVDLKMTSLTTEDTATYFCARNDIYWAFGLWGQGTLVTVSS

SEQ ID NO: 58 - protein, 8 aa, Artificial sequence
  Synthetic amino acid
GFSISTYA

SEQ ID NO: 59 - protein, 7 aa, Artificial sequence
  Synthetic amino acid
IGTGGSA

SEQ ID NO: 60 - protein, 11 aa, Artificial sequence
  Synthetic amino acid
ARNDIYWAFGL

SEQ ID NO: 61 - protein, 111 aa, Artificial sequence
  Synthetic amino acid
ELDLTQTPASVSEPVGGTVTINCQASEGIRNWLAWYQQKPGQPPKLLIYGASTLESGVPSRFKGSGSGTEFTLTIRGVQCDDAATYYCQGGVYSSSIYGYPFGGGTELEIK

SEQ ID NO: 62 - protein, 6 aa, Artificial sequence
  Synthetic amino acid
EGIRNW

SEQ ID NO: 63 - protein, 13 aa, Artificial sequence
  Synthetic amino acid
QGGVYSSSIYGYP

SEQ ID NO: 64 - protein, 123 aa, Artificial sequence
  Synthetic amino acid
QSLEESGGDLVKPGASLTLTCTASGFDFSSSGWICWVRQAPGKGLELIACIYSGRSGSTYYASWAKGRVTISKTSSTTVTLQMTSLTAADTATYFCARALYVDYVDYDYIDLWGPGTLVTVSS

SEQ ID NO: 65 - protein, 9 aa, Artificial sequence
  Synthetic amino acid
GFDFSSSGW

SEQ ID NO: 66 - protein, 9 aa, Artificial sequence
  Synthetic amino acid
IYSGRSGST

SEQ ID NO: 67 - protein, 16 aa, Artificial sequence
  Synthetic amino acid
ARALYVDYVDYDYIDL

SEQ ID NO: 68 - protein, 110 aa, Artificial sequence
  Synthetic amino acid
ELDLTQTPASVEAAVGGTVTIKCQASQSTGIRLAWYQQKPGQPPKLLMYATSNLASGVSSRFKGSGSGTEFTLTISDLECADAATYYCQYSYYGSSYVFDFGGGTEVEIK

SEQ ID NO: 69 - protein, 6 aa, Artificial sequence
  Synthetic amino acid
QSTGIR

SEQ ID NO: 70 - protein, 12 aa, Artificial sequence
  Synthetic amino acid
QYSYYGSSYVFD

SEQ ID NO: 71 - protein, 113 aa, Artificial sequence
  Synthetic amino acid
EQSVEESGGRLVTPGTPLTLTCTASGFSLSSYYMSWVRQAPGRGLEYIGVINTGGSAVYATWTKGRFTISRTSTTVDLKMTGLTTEDTATYFCARGWSRGDLWGQGTLVTISS

SEQ ID NO: 72 - protein, 8 aa, Artificial sequence
  Synthetic amino acid
GFSLSSYY

SEQ ID NO: 73 - protein, 7 aa, Artificial sequence
  Synthetic amino acid
INTGGSA

SEQ ID NO: 74 - protein, 9 aa, Artificial sequence
  Synthetic amino acid
ARGWSRGDL

SEQ ID NO: 75 - protein, 109 aa, Artificial sequence
  Synthetic amino acid
ELDLTQTPASVSEPVGGTVTIKCQASESVDNWLAWYQQKPGQPPKLLIYDASKLASGVPDRFSGSGSGTQFTLTISGVQCDDAATYYCLGVFHDGINNAFGGGTEVEIK

SEQ ID NO: 76 - protein, 6 aa, Artificial sequence
  Synthetic amino acid
ESVDNW

SEQ ID NO: 77 - protein, 11 aa, Artificial sequence
  Synthetic amino acid
LGVFHDGINNA

SEQ ID NO: 78 - protein, 113 aa, Artificial sequence; identical to SEQ ID NO: 71
  Synthetic amino acid

SEQ ID NO: 79 - protein, 8 aa, Artificial sequence
  Synthetic amino acid
GFSLSSYY

SEQ ID NO: 80 - protein, 7 aa, Artificial sequence
  Synthetic amino acid
INTGGSA

SEQ ID NO: 81 - protein, 9 aa, Artificial sequence
  Synthetic amino acid
ARGWSRGDL

SEQ ID NO: 82 - protein, 111 aa, Artificial sequence
  Synthetic amino acid
ELDMTQTPSPVSAAVGGTVTIKCQSSQNVYDDDTLSWYQQKPGQPPKLLIYDASKLASGVPDRFSGSGSGTQFTLTISGVQCDDAATYYCLGVFHDGINNAFGGGTEVEIK

SEQ ID NO: 83 - protein, 8 aa, Artificial sequence
  Synthetic amino acid
QNVYDDDT

SEQ ID NO: 84 - protein, 11 aa, Artificial sequence
  Synthetic amino acid
LGVFHDGINNA

SEQ ID NO: 85 - protein, 117 aa, Artificial sequence
  Synthetic amino acid
EQSVESGGDLVKPEGSLTLTCTVSGFSFSSSYWICWVRQAPGKGLEWIGCIGTGSGSTYYGSWAKGRFTISKTSSTTVTLQMTSLTAADTATYFCVRGAGYSSYRLWGPGTLVTISS

SEQ ID NO: 86 - protein, 9 aa, Artificial sequence
  Synthetic amino acid
GFSFSSSYW

SEQ ID NO: 87 - protein, 7 aa, Artificial sequence
  Synthetic amino acid
IGTGSGS

SEQ ID NO: 88 - protein, 11 aa, Artificial sequence
  Synthetic amino acid
VRGAGYSSYRL

SEQ ID NO: 89 - protein, 110 aa, Artificial sequence
  Synthetic amino acid
ELDMTQTPASVSEPVGGTVTIKCQASESVSNWLAWYQQKPGQRPKLLIYGASTLESGVPSRFSGSGSGTEFTLTISNLECADAATYYCQQGYDWDNIDNAFGGGTEVVVK

SEQ ID NO: 90 - protein, 6 aa, Artificial sequence
  Synthetic amino acid
ESVSNW

SEQ ID NO: 91 - protein, 12 aa, Artificial sequence
  Synthetic amino acid
QQGYDWDNIDNA

SEQ ID NO: 92 - protein, 123 aa, Artificial sequence
  Synthetic amino acid
QSVKESGGDLVKPGASLTLTCTASGFSFISTYWICWVRQAPGKGLELIACIYTGGSGSTYYASWAKGRFTISKTSSTTVTLQLNSLTAADTATYFCARALYVDYVDYDYIDLWGPGTLVTVSS

SEQ ID NO: 93 - protein, 9 aa, Artificial sequence
  Synthetic amino acid
GFSFISTYW

SEQ ID NO: 94 - protein, 9 aa, Artificial sequence
  Synthetic amino acid
IYTGGSGST

SEQ ID NO: 95 - protein, 16 aa, Artificial sequence
  Synthetic amino acid
ARALYVDYVDYDYIDL

SEQ ID NO: 96 - protein, 110 aa, Artificial sequence
  Synthetic amino acid
ELDLTQTPASVEAAVGGTVTIKCQASENIGSRLAWYQQKPGQPPKLLIYAASNLASGVSSRFKGSRSGTQFTLTISDLECADAAIYYCQCSYYGSTYVFGFGGGTEVEIK

SEQ ID NO: 97 - protein, 6 aa, Artificial sequence
  Synthetic amino acid
ENIGSR

SEQ ID NO: 98 - protein, 12 aa, Artificial sequence
  Synthetic amino acid
QCSYYGSTYVFG

SEQ ID NO: 99 - protein, 120 aa, Artificial sequence
  Synthetic amino acid
EQSVEESGGDLVKPGTSLTLTCKMSGFSLSSSYWICWVRQAPGKGLEWIGCIDSGSVGITYYATWAKGRFTISRSTSLNTVTLQMTSLTGADTAMYFSVRHGDNWALDLWGPGTLVTISS

SEQ ID NO: 100 - protein, 9 aa, Artificial sequence
  Synthetic amino acid
GFSLSSSYW

SEQ ID NO: 101 - protein, 9 aa, Artificial sequence
  Synthetic amino acid
IDSGSVGIT

SEQ ID NO: 102 - protein, 12 aa, Artificial sequence
  Synthetic amino acid
SVRHGDNWALDL

SEQ ID NO: 103 - protein, 110 aa, Artificial sequence
  Synthetic amino acid
ELVLTQTPASVSEPVGGTVTIKCQASQSINSWLAWYQQKPGQPPKLLIYKASTLASGVPSRFSASGSGTEFTLTITGVQCDDAATYYCQHGYIRGDLDNVFGGGTEVVVK

SEQ ID NO: 104 - protein, 6 aa, Artificial sequence
  Synthetic amino acid
QSINSW

SEQ ID NO: 105 - protein, 12 aa, Artificial sequence
  Synthetic amino acid
QHGYIRGDLDNV

SEQ ID NO: 106 - DNA, 369 bp, Artificial sequence
  Synthetic nucleic acid
gagcagtcgttggaggagtccgggggtctggaggagtccgggggtcgcctggtcacgcctgggacacccctgacactcacctgcacagcctctggattcaccatcaatagcgcccacatgtcttgggtccgccaggctccagggaaggggctggaatggatcggattcagtactactggtggtccctcatattacgcgaactgggcaaaaggccgattcaccatctccagaacctcgaccacggtggatctggagatcaccagtccgacaatcgaggacacggccacctatttctgtgccagagatggtcctggtaataatattgatatggacttgtggggccaaggcaccctggtcaccatcacctca

SEQ ID NO: 107 - DNA, 24 bp, Artificial sequence
  Synthetic nucleic acid
ggattcaccatcaatagcgcccac

SEQ ID NO: 108 - DNA, 21 bp, Artificial sequence
  Synthetic nucleic acid
agtactactggtggtccctca

SEQ ID NO: 109 - DNA, 39 bp, Artificial sequence
  Synthetic nucleic acid
gccagagatggtcctggtaataatattgatatggacttg

SEQ ID NO: 110 - DNA, 330 bp, Artificial sequence
  Synthetic nucleic acid
gagctcgatctgacccagacaccagcctccgtgtctgaacctgtgggaggcacagtcaccatcaagtgccaggccagtcagaataggggcggtagcatagcctggtatcagcagaaaccagggcagcctcccaagctcctgatctattctgcatccactctggcatctggggtcccatcgcggttcagcggcagtggatatgggacagagttcactctcaccatcagcggcgtgcagtgtgccgatgctggcacttactactgccaatctactatttatagtataagtgatattggggctttcggcggagggaccgaggtggtggtcaaa

SEQ ID NO: 111 - DNA, 18 bp, Artificial sequence
  Synthetic nucleic acid
cagaataggggcggtagc

SEQ ID NO: 112 - DNA, 36 bp, Artificial sequence
  Synthetic nucleic acid
caatctactatttatagtataagtgatattggggct

SEQ ID NO: 113 - DNA, 345 bp, Artificial sequence
  Synthetic nucleic acid
cagtcggtggaggagtccgggggtcgcctggtcacgcctgggacacccctgacactcacctgcacagtctctggaatcgacctcactaactatgcaataaactgggtccgccaggctccaggggaggggctggaatacatcggaaccattactggtagtagtaacacattctacgcgagctgggcgaaaggccgattcaccatctccaaaacctcgaccacggtggatctgaaaatcaccagtccgacaactgaggacacgggcacctatttctgtgccagtaatcctgatagtcacaacgctaatggcgtgtggggccaaggcaccctggtcaccgtctcctca

SEQ ID NO: 114 - DNA, 24 bp, Artificial sequence
  Synthetic nucleic acid
ggaatcgacctcactaactatgca

SEQ ID NO: 115 - DNA, 21 bp, Artificial sequence
  Synthetic nucleic acid
attactggtagtagtaacaca

SEQ ID NO: 116 - DNA, 36 bp, Artificial sequence
  Synthetic nucleic acid
gccagtaatcctgatagtcacaacgctaatggcgtg

SEQ ID NO: 117 - DNA, 336 bp, Artificial sequence
  Synthetic nucleic acid
gagctcgtgatgacccagacaccagcctccgtgtctgaacctgtggaaggcacagtcaccatcaagtgtcaggccagtcagagtgtttatgataacaacttagcctggtatcagcagaaaccagggcagcctcccaagctcctgatctattctgcatccactctggcatctggggtcccatcgcggttcagcggcagtggatatgggacagagttcactctcaccatcagcggcgtggagtgtgccgatgctgccacttactattgtcaaagctatggtattactaataagaataattataatagtttcggcggagggaccgaggtggtggtcaaa

SEQ ID NO: 118 - DNA, 21 bp, Artificial sequence
  Synthetic nucleic acid
cagagtgtttatgataacaac

SEQ ID NO: 119 - DNA, 39 bp, Artificial sequence
  Synthetic nucleic acid
caaagctatggtattactaataagaataattataatagt

SEQ ID NO: 120 - DNA, 363 bp, Artificial sequence
  Synthetic nucleic acid
gagcagtcggtggaggagtccgggggagacctggtcaagcctggggcatccctgacactcacctgcgcagcctctggattctccttcagtagcacctactgcatgtgctgggtccgccaggctccagggaagggcctggagtggatcgcatgcattcatggtgtaagtactaataatagatggtacgcgagctggccgaaaggccgattcaccatctccaaaacctcgtcgaccacggtgactctgcaaatgaccagtctgacagccgcggacacggccacctacttctgtgcgagaagtgacactgactatgagtggggtctttccttgtggggcccaggcaccctggtcaccatctcttca

SEQ ID NO: 121 - DNA, 27 bp, Artificial sequence
  Synthetic nucleic acid
ggattctccttcagtagcacctactgc

SEQ ID NO: 122 - DNA, 27 bp, Artificial sequence
  Synthetic nucleic acid
attcatggtgtaagtactaataataga

SEQ ID NO: 123 - DNA, 39 bp, Artificial sequence
  Synthetic nucleic acid
gcgagaagtgacactgactatgagtggggtctttccttg

SEQ ID NO: 124 - DNA, 324 bp, Artificial sequence
  Synthetic nucleic acid
gagctcgatctgacccagacaccagcctccgtgtctgagcctgtgggaggcacagtcaccatcaagtgccaggccagtgagagcattggtagtagattagcctggtatcaacagaaaccagggcagcgtcccaagctcctgatctacaaggcatccactctggcatctggggtcccatcgcggttcagtggcagtggatctgggacagagttcactctcaccgtcagcgacctggagtgtgccgatgttgccgcttactattgtcaatgcgctggtcagagtagtacttgggctttcggcggagggaccgaggtggaaatcaaa

SEQ ID NO: 125 - DNA, 18 bp, Artificial sequence
  Synthetic nucleic acid
gagagcattggtagtaga

SEQ ID NO: 126 - DNA, 30 bp, Artificial sequence
  Synthetic nucleic acid
caatgcgctggtcagagtagtacttgggct

SEQ ID NO: 127 - DNA, 363 bp, Artificial sequence; identical to SEQ ID NO: 120
  Synthetic nucleic acid

SEQ ID NO: 128 - DNA, 27 bp, Artificial sequence
  Synthetic nucleic acid
ggattctccttcagtagcacctactgc

SEQ ID NO: 129 - DNA, 27 bp, Artificial sequence
  Synthetic nucleic acid
attcatggtgtaagtactaataataga

SEQ ID NO: 130 - DNA, 39 bp, Artificial sequence; identical to SEQ ID NO: 123
  Synthetic nucleic acid

SEQ ID NO: 131 - DNA, 324 bp, Artificial sequence
  Synthetic nucleic acid
gagctcgtgatgacccagacaccagcctccgtggaggcagttgtgggaggcacagtcaccatcaagtgccaggccagtgagagcattggtagtagattagcctggtatcaacagaaaccagggcagcgtcccaagctcctgatctacaaggcatccactctggcatctggggtcccatcgcggttcagtggcagtggatctgggacagagttcactctcaccgtcagcgacctggagtgtgccgatgttgccgcttactattgtcaatgcgctggtcagagtagtacttgggctttcggcggagggaccgaggtggtggtcaaa

SEQ ID NO: 132 - DNA, 18 bp, Artificial sequence
  Synthetic nucleic acid
gagagcattggtagtaga

SEQ ID NO: 133 - DNA, 30 bp, Artificial sequence; identical to SEQ ID NO: 126
  Synthetic nucleic acid

SEQ ID NO: 134 - DNA, 360 bp, Artificial sequence
  Synthetic nucleic acid
cagtcggtgaaggagtccgggggtcgcctggtcacgcctgggacacccctgacactcacctgcaccgtctctggattctccctcagtaacaatggaatgagctgggtccgccaggctccagggaaggggctggagtggatcggaatcatttatgttgggagtggtaccacagactacgcgacctgggcgaaaggccgattcaccatctccagaacctcgaccacggtggatctgaaaatgaccagtctgacaaccgaggacacggccacctatttatgtgccagaggttttggtgttggggattggcaagaatggttttttgatctctggggcccaggcaccctggtcaccatctcttca

SEQ ID NO: 135 - DNA, 24 bp, Artificial sequence
  Synthetic nucleic acid
ggattctccctcagtaacaatgga

SEQ ID NO: 136 - DNA, 24 bp, Artificial sequence
  Synthetic nucleic acid
atttatgttgggagtggtaccaca

SEQ ID NO: 137 - DNA, 48 bp, Artificial sequence
  Synthetic nucleic acid
gccagaggttttggtgttggggattggcaagaatggttttttgatctc

SEQ ID NO: 138 - DNA, 324 bp, Artificial sequence
  Synthetic nucleic acid
gagctcgtgatgacccagacaccagcctccgtgtctgagcctgtgggaggcacagtcaccatcaagtgccaggccagtgaaagcattagcaactacttatcctggtatcagcagaaaccagggcagcctcccaagctcctgatctataaggcatccactctggcatctggggtctcatcgcggttcaaaggcagtggatctgggacagaattcactctcaccatcagcgacctggagtgtgccgatgctgccacttactactgtcaagcctattggggtacttctactatggctttcggcggagggaccgaggtggaaatcaac

SEQ ID NO: 139 - DNA, 18 bp, Artificial sequence
  Synthetic nucleic acid
gaaagcattagcaactac

SEQ ID NO: 140 - DNA, 30 bp, Artificial sequence
  Synthetic nucleic acid
caagcctattggggtacttctactatggct

SEQ ID NO: 141 - DNA, 360 bp, Artificial sequence
  Synthetic nucleic acid
cagtcgttggaggagtccgggggtcgcctggtcacgcctgggacacccctgacactcacctgcaccgtctctggattctccctcagtaacaatggaatgagctgggtccgccaggctccagggaaggggctggagtggatcggaatcatttatgttgggagtggtaccacagactacgcgagctggccgaaaggccgattcaccatctccagaacctcgaccacggtggatctgaaaatgaccagtctgacaaccgaggacacggccacctatttatgtgccagaggttttggtgttggggattggcaagaatggttttttgatctctggggcccaggcaccctggtcaccgtctcttct

SEQ ID NO: 142 - DNA, 24 bp, Artificial sequence
  Synthetic nucleic acid
ggattctccctcagtaacaatgga

SEQ ID NO: 143 - DNA, 24 bp, Artificial sequence
  Synthetic nucleic acid
atttatgttgggagtggtaccaca

SEQ ID NO: 144 - DNA, 48 bp, Artificial sequence; identical to SEQ ID NO: 137
  Synthetic nucleic acid

SEQ ID NO: 145 - DNA, 324 bp, Artificial sequence; identical to SEQ ID NO: 138
  Synthetic nucleic acid

SEQ ID NO: 146 - DNA, 18 bp, Artificial sequence
  Synthetic nucleic acid
gaaagcattagcaactac

SEQ ID NO: 147 - DNA, 30 bp, Artificial sequence; identical to SEQ ID NO: 140
  Synthetic nucleic acid

SEQ ID NO: 148 - DNA, 345 bp, Artificial sequence
  Synthetic nucleic acid
agcagttcggtggaggagtccgggggtcgcctggtcacgcctgggacacccctgacactcacctgcacagtctctggattctccctcagtagctatgcaatggcctgggtccgccaggctccagggaaggggctggaatggatcggaatcattggtactggtaccaccacatactacgcgacctgggtgaatggtcgattcaccatctccaaaacctcgaccacggtggacctgaaaatgaccagtctgacaaccgaggacacggccacttatttctgtgtcagaaatgatgtttattgggcgtttaatttgtggggccaaggcaccctggtcaccgtctcttca

SEQ ID NO: 149 - DNA, 24 bp, Artificial sequence
  Synthetic nucleic acid
ggattctccctcagtagctatgca

SEQ ID NO: 150 - DNA, 21 bp, Artificial sequence
  Synthetic nucleic acid
attggtactggtaccaccaca

SEQ ID NO: 151 - DNA, 33 bp, Artificial sequence
  Synthetic nucleic acid
gtcagaaatgatgtttattgggcgtttaatttg

SEQ ID NO: 152 - DNA, 336 bp, Artificial sequence
  Synthetic nucleic acid
gagctcgtgatgacccagacaccagcccccgtgtctgcagctgtgggaggcacagtcaccatcaactgccaggccagtcagagtgttgttaataataatgccttatcttggtatcagcagaaaccagggcagcctcccaagctcctgatctacaaggcttccactctggcatctggggtcccatcgcggttcaaaggcagtggatctggggcacagttcactctcaccatcagcggcgtgcagtgtgacgatgctgccacttattattgtcaaggcggttattatattggtattagtgactatcctttcggcggcgggaccgaggtggtggtcaaa

SEQ ID NO: 153 - DNA, 24 bp, Artificial sequence
  Synthetic nucleic acid
cagagtgttgttaataataatgcc

SEQ ID NO: 154 - DNA, 36 bp, Artificial sequence
  Synthetic nucleic acid
caaggcggttattatattggtattagtgactatcct

SEQ ID NO: 155 - DNA, 345 bp, Artificial sequence; identical to SEQ ID NO: 148
  Synthetic nucleic acid

SEQ ID NO: 156 - DNA, 24 bp, Artificial sequence
  Synthetic nucleic acid
ggattctccctcagtagctatgca

SEQ ID NO: 157 - DNA, 21 bp, Artificial sequence
  Synthetic nucleic acid
attggtactggtaccaccaca

SEQ ID NO: 158 - DNA, 33 bp, Artificial sequence; identical to SEQ ID NO: 151
  Synthetic nucleic acid

SEQ ID NO: 159 - DNA, 336 bp, Artificial sequence
  Synthetic nucleic acid
gagctcgatctgacccagacaccatcctccgtgtctgcagctgtgggaggcacagtcagcatcagttgccagtccagtcagagtgttgttaataataatgccttatcttggtatcagcagaaaccagggcagcctcccaagctcctgatctacaaggcttccactctggcatctggggtcccatcgcggttcaaaggcagtggatctggggcacagttcactctcaccatcagcggcgtgcagtgtgacgatgctgccacttattattgtcaaggcggttattatattggtattagtgactatcctttcggcggcgggaccgaggtggaaatcaaa

SEQ ID NO: 160 - DNA, 24 bp, Artificial sequence
  Synthetic nucleic acid
cagagtgttgttaataataatgcc

SEQ ID NO: 161 - DNA, 36 bp, Artificial sequence; identical to SEQ ID NO: 154
  Synthetic nucleic acid

SEQ ID NO: 162 - DNA, 345 bp, Artificial sequence
  Synthetic nucleic acid
gagcagtcggtggaggagtccggaggaggcctggtaacgcctggaggaaccctgacactcacctgcacagcctctggattctccatcagtacctatgcaatgatctgggtccgccaggctccaggggaggggctggaatacatcggatgcattggtactggtggtagcgcattctacgcgatctgggcaaaaggccgattcaccatctccagaacctcgaccacggtggatctgaagatgaccagtctgacaaccgaggacacggccacatatttctgtgccagaaatgatatttattgggcctttggcttatggggccaaggcacgctggtcaccgtctcctca

SEQ ID NO: 163 - DNA, 24 bp, Artificial sequence
  Synthetic nucleic acid
ggattctccatcagtacctatgca

SEQ ID NO: 164 - DNA, 21 bp, Artificial sequence
  Synthetic nucleic acid
attggtactggtggtagcgca

SEQ ID NO: 165 - DNA, 33 bp, Artificial sequence
  Synthetic nucleic acid
gccagaaatgatatttattgggcctttggctta

SEQ ID NO: 166 - DNA, 333 bp, Artificial sequence
  Synthetic nucleic acid
gagctcgatctgacccagacaccagcctccgtgtctgaacctgtgggaggcacagtcaccatcaactgccaggccagtgagggcattaggaactggttagcctggtatcagcagaaaccagggcagcctcccaagctcctgatctatggtgcatccactctggaatctggggtcccatcgcggttcaaaggcagtggatctgggacagagttcactctcaccatcagaggtgtgcagtgtgacgatgctgccacttactactgtcaaggcggtgtttatagtagtagtatttatggttatcctttcggcggagggaccgagctggaaatcaaa

SEQ ID NO: 167 - DNA, 18 bp, Artificial sequence
  Synthetic nucleic acid
gagggcattaggaactgg

SEQ ID NO: 168 - DNA, 39 bp, Artificial sequence
  Synthetic nucleic acid
caaggcggtgtttatagtagtagtatttatggttatcct

SEQ ID NO: 169 - DNA, 372 bp, Artificial sequence
  Synthetic nucleic acid
gagcagtcgttggaggagtccgggggagacctggtcaagcctggggcatccctgacactcacctgcacagcctctggattcgactttagtagtagtggttggatatgttgggtccgccaggctccagggaagggactggagttgatcgcatgcatttatagtggtcgcagtggtagcacttactacgcgagctgggcgaaaggccgagtcaccatctccaaaacctcgtcgaccacggtgactctgcagatgaccagtctgacagccgcggacacggccacctatttctgtgcgagagccctctatgttgattatgttgattatgattatatagatttgtggggcccaggcaccctggtcaccgtctcctca

SEQ ID NO: 170 - DNA, 27 bp, Artificial sequence
  Synthetic nucleic acid
ggattcgactttagtagtagtggttgg

SEQ ID NO: 171 - DNA, 27 bp, Artificial sequence
  Synthetic nucleic acid
atttatagtggtcgcagtggtagcact

SEQ ID NO: 172 - DNA, 48 bp, Artificial sequence
  Synthetic nucleic acid
gcgagagccctctatgttgattatgttgattatgattatatagatttg

SEQ ID NO: 173 - DNA, 330 bp, Artificial sequence
  Synthetic nucleic acid
gagctcgatctgacccagactccagcctccgtggaggcagctgtgggaggcacagtcaccatcaagtgccaggccagtcagagcactggtattagattagcctggtatcagcagaaaccagggcagcctcccaaactcctgatgtatgctacatccaatctggcatctggggtctcatcgcggttcaaaggcagtggatctgggacagagttcactctcaccatcagcgacctggagtgtgccgatgctgccacttactactgtcaatatagttattatggtagtagttatgtttttgatttcggcggagggaccgaggtggaaatcaaa

SEQ ID NO: 174 - DNA, 18 bp, Artificial sequence
  Synthetic nucleic acid
cagagcactggtattaga

SEQ ID NO: 175 - DNA, 36 bp, Artificial sequence
  Synthetic nucleic acid
caatatagttattatggtagtagttatgtttttgat

SEQ ID NO: 176 - DNA, 339 bp, Artificial sequence
  Synthetic nucleic acid
gagcagtcggtggaggagtccgggggtcgcctggtcacgcctgggacacccctgacactcacctgcacagcctctggattctccctcagtagctactacatgagctgggtccgccaggctccagggaggggactggaatacatcggagtcattaatactggtggtagcgcagtctacgcgacctggacaaaaggccgattcaccatctccagaacctcgaccacggtggatctgaaaatgaccggtctgacaaccgaggacacggccacctatttctgtgccagaggatggagtaggggtgacttgtggggccaaggcaccctggtcaccatctcctca

SEQ ID NO: 177 - DNA, 24 bp, Artificial sequence
  Synthetic nucleic acid
ggattctccctcagtagctactac

SEQ ID NO: 178 - DNA, 21 bp, Artificial sequence
  Synthetic nucleic acid
attaatactggtggtagcgca

SEQ ID NO: 179 - DNA, 27 bp, Artificial sequence
  Synthetic nucleic acid
gccagaggatggagtaggggtgacttg

SEQ ID NO: 180 - DNA, 327 bp, Artificial sequence
  Synthetic nucleic acid
gagctcgatctgacccagacaccagcctccgtgtctgaacctgtgggaggcacagtcaccatcaagtgccaggccagtgaaagcgttgacaactggttagcctggtatcagcagaaaccagggcagcctcccaaactcctgatctacgatgcatccaaattggcatctggggtcccagataggttcagcggcagtggatctgggacacagttcactctcaccatcagcggcgtgcagtgtgacgatgctgccacttactactgtctaggcgtttttcatgatggtattaataatgctttcggcggagggaccgaggtggaaatcaaa

SEQ ID NO: 181 - DNA, 18 bp, Artificial sequence
  Synthetic nucleic acid
gaaagcgttgacaactgg

SEQ ID NO: 182 - DNA, 33 bp, Artificial sequence
  Synthetic nucleic acid
ctaggcgtttttcatgatggtattaataatgct

SEQ ID NO: 183 - DNA, 339 bp, Artificial sequence; identical to SEQ ID NO: 176
  Synthetic nucleic acid

SEQ ID NO: 184 - DNA, 24 bp, Artificial sequence
  Synthetic nucleic acid
ggattctccctcagtagctactac

SEQ ID NO: 185 - DNA, 21 bp, Artificial sequence
  Synthetic nucleic acid
attaatactggtggtagcgca

SEQ ID NO: 186 - DNA, 27 bp, Artificial sequence
  Synthetic nucleic acid
gccagaggatggagtaggggtgacttg

SEQ ID NO: 187 - DNA, 333 bp, Artificial sequence
  Synthetic nucleic acid
gagctcgatatgacccagacaccatcgcccgtgtctgcagctgtgggaggcacagtcaccatcaagtgccagtccagtcagaatgtttatgatgacgatactttatcctggtatcagcagaaaccagggcagcctcccaaactcctgatctacgatgcatccaaattggcatctggggtcccagataggttcagcggcagtggatctgggacacagttcactctcaccatcagcggcgtgcagtgtgacgatgctgccacttactactgtctaggcgtttttcatgatggtattaataatgctttcggcggagggaccgaggtggaaatcaaa

SEQ ID NO: 188 - DNA, 24 bp, Artificial sequence
  Synthetic nucleic acid
cagaatgtttatgatgacgatact

SEQ ID NO: 189 - DNA, 33 bp, Artificial sequence; identical to SEQ ID NO: 182
  Synthetic nucleic acid

SEQ ID NO: 190 - DNA, 351 bp, Artificial sequence
  Synthetic nucleic acid
gagcagtcggtggagtccgggggagacctggtcaagcctgagggatccctgacactcacctgcacagtctctggattctccttcagtagcagctactggatatgctgggtccgccaggctccagggaaggggctggaatggatcggatgcattggtactggtagtggtagcacttactacgggagctgggcgaaaggccgattcaccatctccaaaacctcgtcgaccacggtgactctgcaaatgaccagtctgacagccgcggacacggccacctatttctgtgtgagaggggctggttatagttcttataggttgtggggcccaggcaccctggtcaccatctcctca

SEQ ID NO: 191 - DNA, 27 bp, Artificial sequence
  Synthetic nucleic acid
ggattctccttcagtagcagctactgg

SEQ ID NO: 192 - DNA, 21 bp, Artificial sequence
  Synthetic nucleic acid
attggtactggtagtggtagc

SEQ ID NO: 193 - DNA, 33 bp, Artificial sequence
  Synthetic nucleic acid
gtgagaggggctggttatagttcttataggttg

SEQ ID NO: 194 - DNA, 330 bp, Artificial sequence
  Synthetic nucleic acid
gagctcgatatgacccagacaccagcctccgtgtctgaacctgtgggaggcacagtcaccatcaagtgccaggccagtgaaagcgttagcaactggttagcctggtatcagcagaaaccagggcagcgtcccaagctcctgatctatggtgcatccactctggaatctggggtcccatcgcggttcagcggcagtggatctgggacagagttcactctcaccatcagcaacctggagtgtgccgatgctgccacttactactgtcaacagggttatgattgggataatatcgataatgctttcggcggagggaccgaggtggtggtcaaa

SEQ ID NO: 195 - DNA, 18 bp, Artificial sequence
  Synthetic nucleic acid
gaaagcgttagcaactgg

SEQ ID NO: 196 - DNA, 36 bp, Artificial sequence
  Synthetic nucleic acid
caacagggttatgattgggataatatcgataatgct

SEQ ID NO: 197 - DNA, 369 bp, Artificial sequence
  Synthetic nucleic acid
cagtcggtgaaggagtccgggggagacctggtcaagcctggggcatccctgacactcacctgcacagcctctggattctccttcattagcacctactggatatgctgggtccgccaggctccagggaaggggctggagttgatcgcatgcatttatactggtggtagtggtagcacttactacgcgagctgggcgaaaggccgattcaccatctccaaaacctcgtcgaccacggtgactctgcaactgaacagtctgacagccgcggacacggccacctatttctgtgcgagagccctctatgttgattatgttgattatgattatatagatttgtggggcccaggcaccctggtcaccgtctcctca

SEQ ID NO: 198 - DNA, 27 bp, Artificial sequence
  Synthetic nucleic acid
ggattctccttcattagcacctactgg

SEQ ID NO: 199 - DNA, 27 bp, Artificial sequence
  Synthetic nucleic acid
atttatactggtggtagtggtagcact

SEQ ID NO: 200 - DNA, 48 bp, Artificial sequence; identical to SEQ ID NO: 172
  Synthetic nucleic acid

SEQ ID NO: 201 - DNA, 330 bp, Artificial sequence
  Synthetic nucleic acid
gagctcgatctgacccagacaccagcctccgtggaggcagctgtgggaggcacagtcaccatcaagtgccaggccagtgagaacattggtagtagattagcctggtatcagcagaaaccagggcagcctcccaagctcctgatctatgctgcatccaatctggcatctggggtctcatcgcggttcaaaggcagtagatctgggacacagttcactctcaccatcagcgacctagagtgtgccgatgctgccatttactactgtcaatgtagttattatggtagtacttatgtttttggtttcggcggagggaccgaggtggaaatcaaa

SEQ ID NO: 202 - DNA, 18 bp, Artificial sequence
  Synthetic nucleic acid
gagaacattggtagtaga

SEQ ID NO: 203 - DNA, 36 bp, Artificial sequence
  Synthetic nucleic acid
caatgtagttattatggtagtacttatgtttttggt

SEQ ID NO: 204 - DNA, 360 bp, Artificial sequence
  Synthetic nucleic acid
gagcagtcggtggaggagtccgggggagacctggtcaagcctgggacatccctgacactcacttgtaaaatgtctggattctccctcagtagcagctattggatatgctgggtccgccaggctccagggaagggactggagtggatcggatgcatcgatagtggtagtgttggtatcacttactacgcgacctgggcgaaaggccgattcaccatctccagaagcaccagcctaaacacggtgactctgcaaatgaccagtctgacaggcgcggacacggccatgtatttctctgtgaggcatggtgataattgggctttggatttgtggggcccaggcaccctggtcaccatctcctca

SEQ ID NO: 205 - DNA, 27 bp, Artificial sequence
  Synthetic nucleic acid
ggattctccctcagtagcagctattgg

SEQ ID NO: 206 - DNA, 27 bp, Artificial sequence
  Synthetic nucleic acid
atcgatagtggtagtgttggtatcact

SEQ ID NO: 207 - DNA, 36 bp, Artificial sequence
  Synthetic nucleic acid
tctgtgaggcatggtgataattgggctttggatttg

SEQ ID NO: 208 - DNA, 330 bp, Artificial sequence
  Synthetic nucleic acid
gagctcgtgctgacccagacaccagcctccgtgtctgagcctgtgggaggcacagtcaccatcaagtgccaggccagtcagagtatcaacagttggttagcctggtatcagcagaaaccaggacagcctcccaagctcctgatctacaaggcgtccactctggcatctggggtcccatcgcggttcagtgccagtggatctgggacagagttcactctcaccatcaccggcgtgcagtgcgacgatgctgccacttactactgtcaacatggctatattcgtggtgatcttgataatgttttcggcggagggaccgaggtggtggtcaaa

SEQ ID NO: 209 - DNA, 18 bp, Artificial sequence
  Synthetic nucleic acid
cagagtatcaacagttgg

SEQ ID NO: 210 - DNA, 36 bp, Artificial sequence
  Synthetic nucleic acid
caacatggctatattcgtggtgatcttgataatgtt

SEQ ID NO: 211 - DNA, 21 bp, Artificial sequence
  Synthetic single guide RNA
gaacgactagttaggcgtgta

SEQ ID NO: 212 - DNA, 20 bp, Artificial sequence
  Synthetic single guide RNA
tgttactatcgcagccctgt

SEQ ID NO: 213 - DNA, 20 bp, Artificial sequence
  Synthetic single guide RNA
gtaggtccccccgtgcactg

SEQ ID NO: 214 - DNA, 20 bp, Artificial sequence
  Synthetic single guide RNA
cctgtgacctcagtgcacgg

SEQ ID NO: 215 - DNA, 19 bp, Artificial sequence
  Synthetic single guide RNA
cttttgggattacctgcgc

SEQ ID NO: 216 - DNA, 20 bp, Artificial sequence
  Synthetic single guide RNA
aactggcactgggtcgcttt

SEQ ID NO: 217 - DNA, 20 bp, Artificial sequence
  Synthetic single guide RNA
taagacctacatcgccagcc

SEQ ID NO: 218 - DNA, 20 bp, Artificial sequence
  Synthetic single guide RNA
gaagaacttgcaccagcgtc

SEQ ID NO: 219 - DNA, 20 bp, Artificial sequence
  Synthetic single guide RNA
gagacttcacactttccgtt

SEQ ID NO: 220 - DNA, 20 bp, Artificial sequence
  Synthetic single guide RNA
tacagtactacaactcaagc

SEQ ID NO: 221 - DNA, 20 bp, Artificial sequence
  Synthetic single guide RNA
cacgcagagcgcgtatgccc

SEQ ID NO: 222 - DNA, 20 bp, Artificial sequence
  Synthetic single guide RNA
tggcaacatcacccgctcca

SEQ ID NO: 223 - protein, 120 aa, Artificial sequence
  Synthetic amino acid
EVQLVESGGGLVQPGGSLRLSCAASGFSLSSSYWICWVRQAPGKGLEWIGSIDSGSVGITYYATWAKGRFTISRDNSKNTLYLQMNSLRAEDTAVYYCVRHGDNWALDLWGQGTLVTVSS

SEQ ID NO: 224 - protein, 11 aa, Artificial sequence
  Synthetic amino acid
VRHGDNWALDL

SEQ ID NO: 225 - protein, 120 aa, Artificial sequence
  Synthetic amino acid
EVQLVESGGGLVQPGGSLRLSCAASGFSLSSSYWICWVRQAPGKGLEWVSSIDSGSVGITYYATWAKGRFTISRDNSKNTLYLQMNSLRAEDTAVYYCVRHGDNWALDLWGQGTLVTVSS

SEQ ID NO: 226 - protein, 120 aa, Artificial sequence
  Synthetic amino acid
EVQLVESGGGLVQPGGSLRLSCAASGFSLSSSYWISWVRQAPGKGLEWIGSIDSGSVGITYYATWAKGRFTISRDNSKNTLYLQMNSLRAEDTAVYYCARHGDNWALDLWGQGTLVTVSS

SEQ ID NO: 227 - protein, 11 aa, Artificial sequence
  Synthetic amino acid
ARHGDNWALDL

SEQ ID NO: 228 - protein, 120 aa, Artificial sequence
  Synthetic amino acid
EVQLVESGGGLVQPGGSLRLSCAASGFSLSSSYWISWVRQAPGKGLEWVSSIDSGSVGITYYATWAKGRFTISRDNSKNTLYLQMNSLRAEDTAVYYCARHGDNWALDLWGQGTLVTVSS

SEQ ID NO: 229 - protein, 120 aa, Artificial sequence
  Synthetic amino acid
EVQLVESGGGLVQPGGSLRLSCAASGFSLSSSYWISWVRQAPGKGLEWIGVIDSGSVGITYYATWAKGRFTISRDNSKNTLYLQMNSLRAEDTAVYYCARHGDNWALDLWGQGTLVTVSS

SEQ ID NO: 230 - protein, 120 aa, Artificial sequence
  Synthetic amino acid
EVQLVESGGGLVQPGGSLRLSCAASGFSLSSSYWISWVRQAPGKGLEWIGSIDSGSVGITYYATSAKGRFTISRDNSKNTLYLQMNSLRAEDTAVYYCARHGDNWALDLWGQGTLVTVSS

SEQ ID NO: 231 - protein, 120 aa, Artificial sequence
  Synthetic amino acid
EVQLVESGGGLVQPGGSLRLSCAASGFSLSSSYWISWVRQAPGKGLEWIGSIDSGSVGITYYATWVKGRFTISRDNSKNTLYLQMNSLRAEDTAVYYCARHGDNWALDLWGQGTLVTVSS

SEQ ID NO: 232 - protein, 110 aa, Artificial sequence
  Synthetic amino acid
DIQMTQSPSTLSASVGDRVTITCQASQSINSWLAWYQQKPGKAPKLLIYKASTLASGVPSRFSGSGSGTEFTLTISSLQPDDFATYYCQHGYIRGDLDNVFGGGTKVEIK

SEQ ID NO: 233 - protein, 7 aa, Artificial sequence
  Synthetic amino acid
KASTLAS

SEQ ID NO: 234 - protein, 11 aa, Artificial sequence
  Synthetic amino acid
HGYIRGDLDNV

SEQ ID NO: 235 - protein, 110 aa, Artificial sequence
  Synthetic amino acid
DLVMTQSPSTLSASVGDRVTITCQASQSINSWLAWYQQKPGKPPKLLIYKASTLASGVSSRFSGSGSGTEFTLTISSLQPDDVATYYCQHGYIRGDLDNVFGGGTKVEIK

SEQ ID NO: 236 - protein, 110 aa, Artificial sequence
  Synthetic amino acid
DIQMTQSPSTLSASVGDRVTITCRASQSINSWLAWYQQKPGKAPKLLIYKASTLASGVPSRFSGSGSGTEFTLTISSLQPDDFATYYCQHGYIRGDLDNVFGGGTKVEIK

SEQ ID NO: 237 - protein, 110 aa, Artificial sequence; identical to SEQ ID NO: 236
  Synthetic amino acid

SEQ ID NO: 238 - protein, 236 aa, Homo sapiens
GPLPKPTLWAEPGSVISWGNSVTIWCQGTLEAREYRLDKEESPAPWDRQNPLEPKNKARFSIPSMTEDYAGRYRCYYRSPVGWSQPSDPLELVMTGAYSKPTLSALPSPLVTSGKSVTLLCQSRSPMDTFLLIKERAAHPLLHLRSEHGAQQHQAEFPMSPVTSVHGGTYRCFSSHGFSHYLLSHPSDPLELIVSGSLEDPRPSPTRSVSTAAGPEDQPLMPTGSVPHSGLRRHWE